European Patent Specification EP 3 733 191 B1, published July 10, 2024. Title: METHODS AND MATERIALS FOR KILLING HIV INFECTED CELLS. Applicant: Mayo Foundation for Medical Education and Research. The sequence listing filed with the application follows.

SEQUENCE LISTING (5 sequences)

SEQ ID NO: 1 - protein, 31 aa, artificial
  Casp8p41 BH3-like peptide
DMNLLDIFIEMEKRVILGEGKLDILKRVCAQ

SEQ ID NO: 2 - protein, 23 aa, artificial
  N-terminal control peptide
MDFSRNLYDIGEQLDSEDLASLK

SEQ ID NO: 3 - DNA, 22 bp, artificial
  Synthetic primer
ttaagcctcaataaagcttgcc

SEQ ID NO: 4 - DNA, 20 bp, artificial
  Synthetic primer
gttcgggcgccactgctaga

SEQ ID NO: 5 - DNA, 26 bp, artificial
  Synthetic probe
ccagagtcacacaacagacgggcaca